European Patent Application EP 4 585 687 A1, published July 16, 2025. Title: Human Antibody of Antigen-Binding Fragment Thereof Against Coronavirus Variants. Applicant: NATIONAL UNIVERSITY CORPORATION KUMAMOTO UNIVERSITY. The sequence listing filed with the application follows.

SEQUENCE LISTING (42 sequences)

SEQ ID NO: 1 - protein, 129 aa, synthetic construct
QVQLVQSGAEVKKPGASVRVSCKASGYSFTASYMHWVRQAPGQGLEWMAIINPGDDNTSYAQKFQGRVTLTRDTSTTTVYMELRSLRSEDTAVYYCTRSTRDYVWGNYRYTPGYYLDYWGQGTLVTVSS

SEQ ID NO: 2 - protein, 107 aa, synthetic construct
DIRMTQSPSSLSASVGDRVTITCRASQTISNYLNWYQQKPGKAPKLLIYAASSLQSGVPSRFSGSGSGTDFTLTISSLQPEDFATYYCQQGYITPITFGQGTRLEIK

SEQ ID NO: 3 - protein, 125 aa, synthetic construct
EVQLVQSGAEVKKPGESLKISCKGSGYIFTNYWIGWVRQMPGKGLEWMGIINPRDSDTRYSPSFQGQVTISTDKSINTAYLQWSSLKASDTAMYYCARQQGGFGDLGAYNWFDPWGQGTLVTVSS

SEQ ID NO: 4 - protein, 110 aa, synthetic construct
QSALTQPPSASGTPGQRVTISCSGSSSNIGSNTVNWYQQLPGTAPKLLIYRDHQRPSGVPDRLSGSKFGTSASLAISGLQSEDEAFYYCAAWDDSLNGWVFGGGTKLTVL

SEQ ID NO: 5 - protein, 124 aa, synthetic construct
EVQLVESGGGVVQPGSSLRLSCAASGFTFRSHAMHWVRQAPGKGLEGVAVIWYDGSNKYYADSVKGRFTISRDNSKNTLYLQMNSLRAEDTAVYYCAREGIAVPGNGADAFDIWGQGTMVTVSS

SEQ ID NO: 6 - protein, 107 aa, synthetic construct
DIQMTQSPSSLSASVGDRVTITCRASQSIGNFLNWYQQKPGKAPKLLIYAASSLQSGVPSRFSGSGSGTDFTLTISSLQPEDFATYYCQQTYSTPYTFGQGTKLEIK

SEQ ID NO: 7 - protein, 117 aa, synthetic construct
EVQLVESGGGLVQPGGSLRLSCAASGIIVSRNYMTWVRQAPGKGLEWVSVIYSGGTTYYADSVKGRFTTSRDDSKNTLYLQMNSLRGDDTAVYYCARDPPHRRGSYWGQGTLVTVSS

SEQ ID NO: 8 - protein, 107 aa, synthetic construct
DILMTQSPSSLSASVGDRVTITCQASQDINKYLNWYQQKPGKAPKLLIYDASNLETGVPSRFSGSGSGTDFSFTISSLQPEDVATYYCQQSDNLPPTFGQGTNVEIK

SEQ ID NO: 9 - protein, 8 aa, synthetic construct
GYSFTASY

SEQ ID NO: 10 - protein, 6 aa, synthetic construct
QTISNY

SEQ ID NO: 11 - protein, 8 aa, synthetic construct
GYIFTNYW

SEQ ID NO: 12 - protein, 8 aa, synthetic construct
SSNIGSNT

SEQ ID NO: 13 - protein, 8 aa, synthetic construct
GFTFRSHA

SEQ ID NO: 14 - protein, 6 aa, synthetic construct
QSIGNF

SEQ ID NO: 15 - protein, 8 aa, synthetic construct
GIIVSRNY

SEQ ID NO: 16 - protein, 6 aa, synthetic construct
QDINKY

SEQ ID NO: 17 - protein, 8 aa, synthetic construct
INPGDDNT

SEQ ID NO: 18 - protein, 8 aa, synthetic construct
INPRDSDT

SEQ ID NO: 19 - protein, 8 aa, synthetic construct
IWYDGSNK

SEQ ID NO: 20 - protein, 7 aa, synthetic construct
IYSGGTT

SEQ ID NO: 21 - protein, 22 aa, synthetic construct
TRSTRDYVWGNYRYTPGYYLDY

SEQ ID NO: 22 - protein, 9 aa, synthetic construct
QQGYITPIT

SEQ ID NO: 23 - protein, 18 aa, synthetic construct
ARQQGGFGDLGAYNWFDP

SEQ ID NO: 24 - protein, 11 aa, synthetic construct
AAWDDSLNGWV

SEQ ID NO: 25 - protein, 17 aa, synthetic construct
AREGIAVPGNGADAFDI

SEQ ID NO: 26 - protein, 9 aa, synthetic construct
QQTYSTPYT

SEQ ID NO: 27 - protein, 11 aa, synthetic construct
ARDPPHRRGSY

SEQ ID NO: 28 - protein, 9 aa, synthetic construct
QQSDNLPPT

SEQ ID NO: 29 - protein, 118 aa, synthetic construct
EVQLVESGGGLIQPGGSLRLSCAASGITVSSNYMSWVRQAPGKGLEWVSLIYSGGSTYYADSVKGRFTISRDNSKNTLYLQMNSLRAEDTAVYYCARDLEEAGGMDVWGQGTTVTVSS

SEQ ID NO: 30 - protein, 108 aa, synthetic construct
DIVMTQSPGTLSLSPGERATLSCRASQSVPSIYLAWYQQRPGQAPRLLIYGASSRATGIPDRFSGSGSGTDFTLTISRLEPEDFAVYYCQQYGSSPGTFGQGTKVEIK

SEQ ID NO: 31 - protein, 119 aa, synthetic construct
EVQLVESGGGLIQPGGSLRLSCAASGLTVSRNYMSWVRQAPGRGLEWVSLIYSGGSTYYADSVKGRFTISRDSSKNTLYLQMNSLRAEDTAVYYCARPIVGARAGMDVWGQGTTVTVSS

SEQ ID NO: 32 - protein, 107 aa, synthetic construct
DIRMTQSPSSLSASVGDRVTITCQASQDISNYLNWYQQKPGKAPKLLIYDASNLETGVPSRFSGSGSGTDFTFTISSLQPEDIATYYCQQYDNLPVTFGQGTRLEIK

SEQ ID NO: 33 - protein, 8 aa, synthetic construct
GITVSSNY

SEQ ID NO: 34 - protein, 7 aa, synthetic construct
QSVPSIY

SEQ ID NO: 35 - protein, 8 aa, synthetic construct
GLTVSRNY

SEQ ID NO: 36 - protein, 6 aa, synthetic construct
QDISNY

SEQ ID NO: 37 - protein, 7 aa, synthetic construct
IYSGGST

SEQ ID NO: 38 - protein, 12 aa, synthetic construct
ARDLEEAGGMDV

SEQ ID NO: 39 - protein, 9 aa, synthetic construct
QQYGSSPGT

SEQ ID NO: 40 - protein, 13 aa, synthetic construct
ARPIVGARAGMDV

SEQ ID NO: 41 - protein, 9 aa, synthetic construct
QQYDNLPVT

SEQ ID NO: 42 - protein, 1273 aa, synthetic construct
MFVFLVLLPLVSSQCVNLTTRTQLPPAYTNSFTRGVYYPDKVFRSSVLHSTQDLFLPFFSNVTWFHAIHVSGTNGTKRFDNPVLPFNDGVYFASTEKSNIIRGWIFGTTLDSKTQSLLIVNNATNVVIKVCEFQFCNDPFLGVYYHKNNKSWMESEFRVYSSANNCTFEYVSQPFLMDLEGKQGNFKNLREFVFKNIDGYFKIYSKHTPINLVRDLPQGFSALEPLVDLPIGINITRFQTLLALHRSYLTPGDSSSGWTAGAAAYYVGYLQPRTFLLKYNENGTITDAVDCALDPLSETKCTLKSFTVEKGIYQTSNFRVQPTESIVRFPNITNLCPFGEVFNATRFASVYAWNRKRISNCVADYSVLYNSASFSTFKCYGVSPTKLNDLCFTNVYADSFVIRGDEVRQIAPGQTGKIADYNYKLPDDFTGCVIAWNSNNLDSKVGGNYNYLYRLFRKSNLKPFERDISTEIYQAGSTPCNGVEGFNCYFPLQSYGFQPTNGVGYQPYRVVVLSFELLHAPATVCGPKKSTNLVKNKCVNFNFNGLTGTGVLTESNKKFLPFQQFGRDIADTTDAVRDPQTLEILDITPCSFGGVSVITPGTNTSNQVAVLYQDVNCTEVPVAIHADQLTPTWRVYSTGSNVFQTRAGCLIGAEHVNNSYECDIPIGAGICASYQTQTNSPRRARSVASQSIIAYTMSLGAENSVAYSNNSIAIPTNFTISVTTEILPVSMTKTSVDCTMYICGDSTECSNLLLQYGSFCTQLNRALTGIAVEQDKNTQEVFAQVKQIYKTPPIKDFGGFNFSQILPDPSKPSKRSFIEDLLFNKVTLADAGFIKQYGDCLGDIAARDLICAQKFNGLTVLPPLLTDEMIAQYTSALLAGTITSGWTFGAGAALQIPFAMQMAYRFNGIGVTQNVLYENQKLIANQFNSAIGKIQDSLSSTASALGKLQDVVNQNAQALNTLVKQLSSNFGAISSVLNDILSRLDKVEAEVQIDRLITGRLQSLQTYVTQQLIRAAEIRASANLAATKMSECVLGQSKRVDFCGKGYHLMSFPQSAPHGVVFLHVTYVPAQEKNFTTAPAICHDGKAHFPREGVFVSNGTHWFVTQRNFYEPQIITTDNTFVSGNCDVVIGIVNNTVYDPLQPELDSFKEELDKYFKNHTSPDVDLGDISGINASVVNIQKEIDRLNEVAKNLNESLIDLQELGKYEQYIKWPWYIWLGFIAGLIAIVMVTIMLCCMTSCCSCLKGCCSCGSCCKFDEDDSEPVLKGVKLHYT